European Patent Application EP 4 736 883 A1, published May 6, 2026. Title: 用于预防和治疗病毒感染的偶联物及其用途. Applicant: 上海爱科百发生物医药技术股份有限公司. The sequence listing filed with the application follows.

SEQUENCE LISTING (85 sequences)

SEQ ID NO: 1 - protein, 252 aa, synthetic construct
MYRMQLLSCIALSLALVTNSPRGPTIKPCPPCKCPAPNLLGGPSVFIFPPKIKDVLMISLSPIVTCVVVDVSEDDPDVQISWFVNNVEVHTAQTQTHREDYNSTLRVVSALPIQHQDWMSGKEFKCKVNNKDLPAPIERTISKPKGSVRAPQVYVLPPPEEEMTKKQVTLTCMVTDFMPEDIYVEWTNNGKTELNYKNTEPVLDSDGSYFMYSKLRVEKKNWVERNSYSCSVVHEGLHNHHTTKSFSRTPGK

SEQ ID NO: 2 - protein, 232 aa, synthetic construct
PRGPTIKPCPPCKCPAPNLLGGPSVFIFPPKIKDVLMISLSPIVTCVVVDVSEDDPDVQISWFVNNVEVHTAQTQTHREDYNSTLRVVSALPIQHQDWMSGKEFKCKVNNKDLPAPIERTISKPKGSVRAPQVYVLPPPEEEMTKKQVTLTCMVTDFMPEDIYVEWTNNGKTELNYKNTEPVLDSDGSYFMYSKLRVEKKNWVERNSYSCSVVHEGLHNHHTTKSFSRTPGK

SEQ ID NO: 3 - protein, 251 aa, synthetic construct
MYRMQLLSCIALSLALVTNSMVRSDKTHTCPPCPAPELLGGPSVFLFPPKPKDTLMISRTPEVTCVVVDVSHEDPEVKFNWYVDGVEVHNAKTKPREEQYNSTYRVVSVLTVLHQDWLNGKEYKCKVSNKALPAPIEKTISKAKGQPREPQVYTLPPSREEMTKNQVSLTCLVKGFYPSDIAVEWESNGQPENNYKTTPPVLDSDGSFFLYSKLTVDKSRWQQGNVFSCSVMHEALHNHYTQKSLSLSPGK

SEQ ID NO: 4 - protein, 231 aa, synthetic construct
MVRSDKTHTCPPCPAPELLGGPSVFLFPPKPKDTLMISRTPEVTCVVVDVSHEDPEVKFNWYVDGVEVHNAKTKPREEQYNSTYRVVSVLTVLHQDWLNGKEYKCKVSNKALPAPIEKTISKAKGQPREPQVYTLPPSREEMTKNQVSLTCLVKGFYPSDIAVEWESNGQPENNYKTTPPVLDSDGSFFLYSKLTVDKSRWQQGNVFSCSVMHEALHNHYTQKSLSLSPGK

SEQ ID NO: 5 - protein, 258 aa, synthetic construct
MYRMQLLSCIALSLALVTNSPRGPTIKPCPPCKCPAPNLLGGPSVFIFPPKIKDVLMISLSPIVTCVVVDVSEDDPDVQISWFVNNVEVHTAQTQTHREDYNSTLRVVSALPIQHQDWMSGKEFKCKVNNKDLPAPIERTISKPKGSVRAPQVYVLPPPEEEMTKKQVTLTCMVTDFMPEDIYVEWTNNGKTELNYKNTEPVLDSDGSYFMYSKLRVEKKNWVERNSYSCSVVHEGLHNHHTTKSFSRTPGKHHHHHH

SEQ ID NO: 6 - protein, 238 aa, synthetic construct
PRGPTIKPCPPCKCPAPNLLGGPSVFIFPPKIKDVLMISLSPIVTCVVVDVSEDDPDVQISWFVNNVEVHTAQTQTHREDYNSTLRVVSALPIQHQDWMSGKEFKCKVNNKDLPAPIERTISKPKGSVRAPQVYVLPPPEEEMTKKQVTLTCMVTDFMPEDIYVEWTNNGKTELNYKNTEPVLDSDGSYFMYSKLRVEKKNWVERNSYSCSVVHEGLHNHHTTKSFSRTPGKHHHHHH

SEQ ID NO: 7 - protein, 257 aa, synthetic construct
MYRMQLLSCIALSLALVTNSMVRSDKTHTCPPCPAPELLGGPSVFLFPPKPKDTLMISRTPEVTCVVVDVSHEDPEVKFNWYVDGVEVHNAKTKPREEQYNSTYRVVSVLTVLHQDWLNGKEYKCKVSNKALPAPIEKTISKAKGQPREPQVYTLPPSREEMTKNQVSLTCLVKGFYPSDIAVEWESNGQPENNYKTTPPVLDSDGSFFLYSKLTVDKSRWQQGNVFSCSVMHEALHNHYTQKSLSLSPGKHHHHHH

SEQ ID NO: 8 - protein, 237 aa, synthetic construct
MVRSDKTHTCPPCPAPELLGGPSVFLFPPKPKDTLMISRTPEVTCVVVDVSHEDPEVKFNWYVDGVEVHNAKTKPREEQYNSTYRVVSVLTVLHQDWLNGKEYKCKVSNKALPAPIEKTISKAKGQPREPQVYTLPPSREEMTKNQVSLTCLVKGFYPSDIAVEWESNGQPENNYKTTPPVLDSDGSFFLYSKLTVDKSRWQQGNVFSCSVMHEALHNHYTQKSLSLSPGKHHHHHH

SEQ ID NO: 9 - protein, 262 aa, synthetic construct
MYRMQLLSCIALSLALVTNSMVRSDKTHTCPPCPPCKCPAPELLGGPSVFLFPPKPKDTLMISRTPEVTCVVVDVSHEDPEVKFNWYVDGVEVHNAKTKPREEQYNSTYRVVSVLTVLHQDWLNGKEYKCKVSNKALPAPIEKTISKAKGQPREPQVYTLPPSREEMTKNQVSLTCLVKGFYPSDIAVEWESNGQPENNYKTTPPVLDSDGSFFLYSKLTVDKSRWQQGNVFSCSVMHEALHNHYTQKSLSLSPGKHHHHHH

SEQ ID NO: 10 - protein, 242 aa, synthetic construct
MVRSDKTHTCPPCPPCKCPAPELLGGPSVFLFPPKPKDTLMISRTPEVTCVVVDVSHEDPEVKFNWYVDGVEVHNAKTKPREEQYNSTYRVVSVLTVLHQDWLNGKEYKCKVSNKALPAPIEKTISKAKGQPREPQVYTLPPSREEMTKNQVSLTCLVKGFYPSDIAVEWESNGQPENNYKTTPPVLDSDGSFFLYSKLTVDKSRWQQGNVFSCSVMHEALHNHYTQKSLSLSPGKHHHHHH

SEQ ID NO: 11 - protein, 237 aa, synthetic construct
MVRSDKTHTCPPCPPCKCPAPELLGGPSVFLFPPKPKDTLMISRTPEVTCVVVDVSHEDPEVKFNWYVDGVEVHNAKTKPREEQYNSTYRVVSVLTVLHQDWLNGKEYKCKVSNKALPAPIEKTISKAKGQPREPQVYTLPPSREEMTKNQVSLTCLVKGFYPSDIAVEWESNGQPENNYKTTPPVLDSDGSFFLYSKLTVDKSRWQMQGNVFSCSVMHEALHNHYTQKSLSLSPGK

SEQ ID NO: 12 - protein, 258 aa, synthetic construct
MYRMQLLSCIALSLALVTNSPRGPTIKPCPPCKCPAPNLLGGPSVFIFPPKIKDVLMISLSPIVTCVVVDVSEDDPDVQISWFVNNVEVHTAQTQTHREDYASTLRVVSALPIQHQDWMSGKEFKCKVNNKDLPAPIERTISKPKGSVRAPQVYVLPPPEEEMTKKQVTLTCMVTDFMPEDIYVEWTNNGKTELNYKNTEPVLDSDGSYFMYSKLRVEKKNWVERNSYSCSVVHEGLHNHHTTKSFSRTPGKHHHHHH

SEQ ID NO: 13 - protein, 238 aa, synthetic construct
PRGPTIKPCPPCKCPAPNLLGGPSVFIFPPKIKDVLMISLSPIVTCVVVDVSEDDPDVQISWFVNNVEVHTAQTQTHREDYASTLRVVSALPIQHQDWMSGKEFKCKVNNKDLPAPIERTISKPKGSVRAPQVYVLPPPEEEMTKKQVTLTCMVTDFMPEDIYVEWTNNGKTELNYKNTEPVLDSDGSYFMYSKLRVEKKNWVERNSYSCSVVHEGLHNHHTTKSFSRTPGKHHHHHH

SEQ ID NO: 14 - protein, 257 aa, synthetic construct
MYRMQLLSCIALSLALVTNSMVRSDKTHTCPPCPAPELLGGPSVFLFPPKPKDTLMISRTPEVTCVVVDVSHEDPEVKFNWYVDGVEVHNAKTKPREEQYASTYRVVSVLTVLHQDWLNGKEYKCKVSNKALPAPIEKTISKAKGQPREPQVYTLPPSREEMTKNQVSLTCLVKGFYPSDIAVEWESNGQPENNYKTTPPVLDSDGSFFLYSKLTVDKSRWQQGNVFSCSVMHEALHNHYTQKSLSLSPGKHHHHHH

SEQ ID NO: 15 - protein, 237 aa, synthetic construct
MVRSDKTHTCPPCPAPELLGGPSVFLFPPKPKDTLMISRTPEVTCVVVDVSHEDPEVKFNWYVDGVEVHNAKTKPREEQYASTYRVVSVLTVLHQDWLNGKEYKCKVSNKALPAPIEKTISKAKGQPREPQVYTLPPSREEMTKNQVSLTCLVKGFYPSDIAVEWESNGQPENNYKTTPPVLDSDGSFFLYSKLTVDKSRWQQGNVFSCSVMHEALHNHYTQKSLSLSPGKHHHHHH

SEQ ID NO: 16 - protein, 252 aa, synthetic construct
MKWVTFISLLFLFSSAYSISAMVRSDKTHTCPPCPAPELLGGPSVFLFPPKPKDTLMISRTPEVTCVVVDVSHEDPEVKFNWYVDGVEVHNAKTKPREEQYNSTYRVVSVLTVLHQDWLNGKEYKCKVSNKALPAPIEKTISKAKGQPREPQVYTLPPSREEMTKNQVSLTCLVKGFYPSDIAVEWESNGQPENNYKTTPPVLDSDGSFFLYSKLTVDKSRWQQGNVFSCSVMHEALHNHYTQKSLSLSPGK

SEQ ID NO: 17 - protein, 266 aa, synthetic construct
MKWVTFISLLFLFSSAYSISAMVRSDKTHTCPPCPAPELLGGPSVFLFPPKPKDTLMISRTPEVTCVVVDVSHEDPEVKFNWYVDGVEVHNAKTKPREEQYNSTYRVVSVLTVLHQDWLNGKEYKCKVSNKALPAPIEKTISKAKGQPREPQVYTLPPSREEMTKNQVSLTCLVKGFYPSDIAVEWESNGQPENNYKTTPPVLDSDGSFFLYSKLTVDKSRWQQGNVFSCSVMHEALHNHYTQKSLSLSPGGGGGSEQKLISEEDL

SEQ ID NO: 18 - protein, 248 aa, synthetic construct
ISAMVRSDKTHTCPPCPAPELLGGPSVFLFPPKPKDTLMISRTPEVTCVVVDVSHEDPEVKFNWYVDGVEVHNAKTKPREEQYNSTYRVVSVLTVLHQDWLNGKEYKCKVSNKALPAPIEKTISKAKGQPREPQVYTLPPSREEMTKNQVSLTCLVKGFYPSDIAVEWESNGQPENNYKTTPPVLDSDGSFFLYSKLTVDKSRWQQGNVFSCSVMHEALHNHYTQKSLSLSPGGGGGSEQKLISEEDL

SEQ ID NO: 19 - protein, 252 aa, synthetic construct
MKWVTFISLLFLFSSAYSISAMVRSDKTHTCPPCPAPELLGGPSVFLFPPKPSDTLMISRTPEVTCVVVDVSHEDPEVKFNWYVDGVEVHNAKTKPREEQYNSTYRVVSVLTVLHQDWLNGKEYKCKVSNKALPAPIEKTISKAKGQPREPQVYTLPPSREEMTKNQVSLTCLVKGFYPSDIAVEWESNGQPENNYKTTPPVLDSDGSFFLYSKLTVDKSRWQQGNVFSCSVMHEALHNHYTQKSLSLSPGK

SEQ ID NO: 20 - protein, 234 aa, synthetic construct
ISAMVRSDKTHTCPPCPAPELLGGPSVFLFPPKPSDTLMISRTPEVTCVVVDVSHEDPEVKFNWYVDGVEVHNAKTKPREEQYNSTYRVVSVLTVLHQDWLNGKEYKCKVSNKALPAPIEKTISKAKGQPREPQVYTLPPSREEMTKNQVSLTCLVKGFYPSDIAVEWESNGQPENNYKTTPPVLDSDGSFFLYSKLTVDKSRWQQGNVFSCSVMHEALHNHYTQKSLSLSPGK

SEQ ID NO: 21 - protein, 266 aa, synthetic construct
MKWVTFISLLFLFSSAYSISAMVRSDKTHTCPPCPAPELLGGPSVFLFPPKPSDTLMISRTPEVTCVVVDVSHEDPEVKFNWYVDGVEVHNAKTKPREEQYNSTYRVVSVLTVLHQDWLNGKEYKCKVSNKALPAPIEKTISKAKGQPREPQVYTLPPSREEMTKNQVSLTCLVKGFYPSDIAVEWESNGQPENNYKTTPPVLDSDGSFFLYSKLTVDKSRWQQGNVFSCSVMHEALHNHYTQKSLSLSPGGGGGSEQKLISEEDL

SEQ ID NO: 22 - protein, 248 aa, synthetic construct
ISAMVRSDKTHTCPPCPAPELLGGPSVFLFPPKPSDTLMISRTPEVTCVVVDVSHEDPEVKFNWYVDGVEVHNAKTKPREEQYNSTYRVVSVLTVLHQDWLNGKEYKCKVSNKALPAPIEKTISKAKGQPREPQVYTLPPSREEMTKNQVSLTCLVKGFYPSDIAVEWESNGQPENNYKTTPPVLDSDGSFFLYSKLTVDKSRWQQGNVFSCSVMHEALHNHYTQKSLSLSPGGGGGSEQKLISEEDL

SEQ ID NO: 23 - protein, 266 aa, synthetic construct
MKWVTFISLLFLFSSAYSISAMVRSDKTHTCPPCPAPELLGGPSVFLFPPKPKDTLMISRTPEVTCVVVDVSHEDPEVKFNWYVDGVEVHNAKTKPREEQYASTYRVVSVLTVLHQDWLNGKEYKCKVSNKALPAPIEKTISKAKGQPREPQVYTLPPSREEMTKNQVSLTCLVKGFYPSDIAVEWESNGQPENNYKTTPPVLDSDGSFFLYSKLTVDKSRWQQGNVFSCSVMHEALHNHYTQKSLSLSPGGGGGSEQKLISEEDL

SEQ ID NO: 24 - protein, 248 aa, synthetic construct
ISAMVRSDKTHTCPPCPAPELLGGPSVFLFPPKPKDTLMISRTPEVTCVVVDVSHEDPEVKFNWYVDGVEVHNAKTKPREEQYASTYRVVSVLTVLHQDWLNGKEYKCKVSNKALPAPIEKTISKAKGQPREPQVYTLPPSREEMTKNQVSLTCLVKGFYPSDIAVEWESNGQPENNYKTTPPVLDSDGSFFLYSKLTVDKSRWQQGNVFSCSVMHEALHNHYTQKSLSLSPGGGGGSEQKLISEEDL

SEQ ID NO: 25 - protein, 266 aa, synthetic construct
MKWVTFISLLFLFSSAYSISAMVRSDKTHTCPPCPAPELLGGPSVFLFPPKPKDTLMISRTPEVTCVVVDVSHEDPEVKFNWYVDGVEVHNAKTKPREEQYNSTYRVVSVLTVLAQDWLNGKEYKCKVSNKALPAPIEKTISKAKGQPREPQVYTLPPSREEMTKNQVSLTCLVKGFYPSDIAVEWESNGQPENNYKTTPPVLDSDGSFFLYSKLTVDKSRWQQGNVFSCSVMHEALHNAYTQKSLSLSPGGGGGSEQKLISEEDL

SEQ ID NO: 26 - protein, 248 aa, synthetic construct
ISAMVRSDKTHTCPPCPAPELLGGPSVFLFPPKPKDTLMISRTPEVTCVVVDVSHEDPEVKFNWYVDGVEVHNAKTKPREEQYNSTYRVVSVLTVLAQDWLNGKEYKCKVSNKALPAPIEKTISKAKGQPREPQVYTLPPSREEMTKNQVSLTCLVKGFYPSDIAVEWESNGQPENNYKTTPPVLDSDGSFFLYSKLTVDKSRWQQGNVFSCSVMHEALHNAYTQKSLSLSPGGGGGSEQKLISEEDL

SEQ ID NO: 27 - protein, 266 aa, synthetic construct
MKWVTFISLLFLFSSAYSISAMVRSDKTHTCPPCPAPELLGGPSVFLFPPKPKDTLMISRTPEVTCVVVDVSHEDPEVKFNWYVDGVEVHNAKTKPREEQYNSTYRVVSVLTVLHQDWLNGKEYKCKVSNKALPAPIEKTISKAKGQPREPQVYTLPPSREEMTKNQVSLTCLVKGFYPSDIAVEWESNGQPENNYKTTPPVLDSDGSFFLYSKLTVDKSRWQQGNVFSCSVMHEALHNHYTQKSLSLSPGGGGGSEQFLISEEDL

SEQ ID NO: 28 - protein, 248 aa, synthetic construct
ISAMVRSDKTHTCPPCPAPELLGGPSVFLFPPKPKDTLMISRTPEVTCVVVDVSHEDPEVKFNWYVDGVEVHNAKTKPREEQYNSTYRVVSVLTVLHQDWLNGKEYKCKVSNKALPAPIEKTISKAKGQPREPQVYTLPPSREEMTKNQVSLTCLVKGFYPSDIAVEWESNGQPENNYKTTPPVLDSDGSFFLYSKLTVDKSRWQQGNVFSCSVMHEALHNHYTQKSLSLSPGGGGGSEQFLISEEDL

SEQ ID NO: 29 - protein, 266 aa, synthetic construct
MKWVTFISLLFLFSSAYSISAMVRSDKTHTCPPCPAPELLGGPSVFLFPPKPKDTLMISRTPEVTCVVVDVSHEDPEVKFNWYVDGVEVHNAKTKPREEQYASTYRVVSVLTVLHQDWLNGKEYKCKVSNKALPAPIEKTISKAKGQPREPQVYTLPPSREEMTKNQVSLTCLVKGFYPSDIAVEWESNGQPENNYKTTPPVLDSDGSFFLYSKLTVDKSRWQQGNVFSCSVMHEALHNHYTQKSLSLSPGGGGGSEQFLISEEDL

SEQ ID NO: 30 - protein, 248 aa, synthetic construct
ISAMVRSDKTHTCPPCPAPELLGGPSVFLFPPKPKDTLMISRTPEVTCVVVDVSHEDPEVKFNWYVDGVEVHNAKTKPREEQYASTYRVVSVLTVLHQDWLNGKEYKCKVSNKALPAPIEKTISKAKGQPREPQVYTLPPSREEMTKNQVSLTCLVKGFYPSDIAVEWESNGQPENNYKTTPPVLDSDGSFFLYSKLTVDKSRWQQGNVFSCSVMHEALHNHYTQKSLSLSPGGGGGSEQFLISEEDL

SEQ ID NO: 31 - protein, 259 aa, synthetic construct
MKWVTFISLLFLFSSAYSDKTHTCPPCPAPELLGGPSVFLFPPKPKDTLMISRTPEVTCVVVDVSHEDPEVKFNWYVDGVEVHNAKTKPREEQYNSTYRVVSVLTVLHQDWLNGKEYKCKVSNKALPAPIEKTISKAKGQPREPQVYTLPPSRDELTKNQVSLTCLVKGFYPSDIAVEWESNGQPENNYKTTPPVLDSDGSFFLYSKLTVDKSRWQQGNVFSCSVMHEALHNHYTQKSLSLSPGGGGGSEQFLISEEDL

SEQ ID NO: 32 - protein, 245 aa, synthetic construct
MKWVTFISLLFLFSSAYSDKTHTCPPCPAPELLGGPSVFLFPPKPKDTLMISRTPEVTCVVVDVSHEDPEVKFNWYVDGVEVHNAKTKPREEQYNSTYRVVSVLTVLHQDWLNGKEYKCKVSNKALPAPIEKTISKAKGQPREPQVYTLPPSRDELTKNQVSLTCLVKGFYPSDIAVEWESNGQPENNYKTTPPVLDSDGSFFLYSKLTVDKSRWQQGNVFSCSVMHEALHNHYTQKSLSLSPGK

SEQ ID NO: 33 - protein, 231 aa, synthetic construct
MVRSDKTHTCPPCPAPELLGGPSVFLFPPKPKDTLYITREPEVTCVVVDVSHEDPEVKFNWYVDGVEVHNAKTKPREEQYNSTYRVVSVLTVLHQDWLNGKEYKCKVSNKALPAPIEKTISKAKGQPREPQVYTLPPSREEMTKNQVSLTCLVKGFYPSDIAVEWESNGQPENNYKTTPPVLDSDGSFFLYSKLTVDKSRWQQGNVFSCSVMHEALHNHYTQKSLSLSPGK

SEQ ID NO: 34 - protein, 250 aa, synthetic construct
MKWVTFISLLFLFSSAYSEPKSSDKTHTCPPCPAPELLGGPSVFLFPPKPKDTLMISRTPEVTCVVVDVSHEDPEVKFNWYVDGVEVHNAKTKPREEQYNSTYRVVSVLTVLHQDWLNGKEYKCKVSNKALPAPIEKTISKAKGQPREPQVYTLPPSRDELTKNQVSLTCLVKGFYPSDIAVEWESNGQPENNYKTTPPVLDSDGSFFLYSKLTVDKSRWQQGNVFSCSVMHEALHNHYTQKSLSLSPGK

SEQ ID NO: 35 - protein, 245 aa, synthetic construct
MGWSCIILFLVATATGVHSKTHTCPPCPAPELLGGPSVFLFPPKPKDTLMISRTPEVTCVVVDVSHEDPEVKFNWYVDGVEVHNAKTKPREEQYNSTYRVVSVLTVLHQDWLNGKEYKCKVSNKALPAPIEKTISKAKGQPREPQVYTLPPSRDELTKNQVSLTCLVKGFYPSDIAVEWESNGQPENNYKTTPPVLDSDGSFFLYSKLTVDKSRWQQGNVFSCSVMHEALHNHYTQKSLSLSPGK

SEQ ID NO: 36 - protein, 226 aa, synthetic construct
KTHTCPPCPAPELLGGPSVFLFPPKPKDTLYITREPEVTCVVVDVSHEDPEVKFNWYVDGVEVHNAKTKPREEQYNSTYRVVSVLTVLHQDWLNGKEYKCKVSNKALPAPIEKTISKAKGQPREPQVYTLPPSRDELTKNQVSLTCLVKGFYPSDIAVEWESNGQPENNYKTTPPVLDSDGSFFLYSKLTVDKSRWQQGNVFSCSVMHEALHNHYTQKSLSLSPGK

SEQ ID NO: 37 - protein, 226 aa, synthetic construct
KTHTCPPCPAPELLGGPSVFLFPPKPKDTLMISRTPEVTCVVVDVSHEDPEVKFNWYVDGVEVHNAKTKPREEQYNSTYRVVSVLTVLHQDWLNGKEYKCKVSNKALPAPIEKTISKAKGQPREPQVYTLPPSRDELTKNQVSLTCLVKGFYPSDIAVEWESNGQPENNYKTTPPVLDSDGSFFLYSKLTVDKSRWQQGNVFSCSVLHEALHSHYTQKSLSLSPGK

SEQ ID NO: 38 - protein, 259 aa, synthetic construct
MKWVTFISLLFLFSSAYSDKTHTCPPCPAPELLGGPSVFLFPPKPKDTLYITREPEVTCVVVDVSHEDPEVKFNWYVDGVEVHNAKTKPREEQYNSTYRVVSVLTVLHQDWLNGKEYKCKVSNKALPAPIEKTISKAKGQPREPQVYTLPPSRDELTKNQVSLTCLVKGFYPSDIAVEWESNGQPENNYKTTPPVLDSDGSFFLYSKLTVDKSRWQQGNVFSCSVMHEALHNHYTQKSLSLSPGGGGGSEQKLISEEDL

SEQ ID NO: 39 - protein, 226 aa, synthetic construct
DKTHTCPPCPAPELLGGPSVFLFPPKPKDTLXIXRXPEVTCVVVDVSHEDPEVKFNWYVDGVEVHNAKTKPREEQYNSTYRVVSVLTVLHQDWLNGKEYKCKVSNKALPAPIEKTISKAKGQPREPQVYTLPPSRXEXTKNQVSLTCLVKGFYPSDIAVEWESNGQPENNYKTTPPVLDSDGSFFLYSKLTVDKSRWQQGNVFSCSVXHEALHXHYTQKSLSLSPG

SEQ ID NO: 40 - protein, 226 aa, synthetic construct
DKTHTCPPCPAPELLGGPSVFLFPPKPKDTLMISRTPEVTCVVVDVSHEDPEVKFNWYVDGVEVHNAKTKPREEQYNSTYRVVSVLTVLHQDWLNGKEYKCKVSNKALPAPIEKTISKAKGQPREPQVYTLPPSRXEXTKNQVSLTCLVKGFYPSDIAVEWESNGQPENNYKTTPPVLDSDGSFFLYSKLTVDKSRWQQGNVFSCSVMHEALHNHYTQKSLSLSPG

SEQ ID NO: 41 - protein, 226 aa, synthetic construct
DKTHTCPPCPAPELLGGPSVFLFPPKPKDTLYITREPEVTCVVVDVSHEDPEVKFNWYVDGVEVHNAKTKPREEQYNSTYRVVSVLTVLHQDWLNGKEYKCKVSNKALPAPIEKTISKAKGQPREPQVYTLPPSRXEXTKNQVSLTCLVKGFYPSDIAVEWESNGQPENNYKTTPPVLDSDGSFFLYSKLTVDKSRWQQGNVFSCSVMHEALHNHYTQKSLSLSPG

SEQ ID NO: 42 - protein, 226 aa, synthetic construct
DKTHTCPPCPAPELLGGPSVFLFPPKPKDTLYITREPEVTCVVVDVSHEDPEVKFNWYVDGVEVHNAKTKPREEQYNSTYRVVSVLTVLHQDWLNGKEYKCKVSNKALPAPIEKTISKAKGQPREPQVYTLPPSRDELTKNQVSLTCLVKGFYPSDIAVEWESNGQPENNYKTTPPVLDSDGSFFLYSKLTVDKSRWQQGNVFSCSVMHEALHNHYTQKSLSLSPG

SEQ ID NO: 43 - protein, 226 aa, synthetic construct
DKTHTCPPCPAPELLGGPSVFLFPPKPKDTLYITREPEVTCVVVDVSHEDPEVKFNWYVDGVEVHNAKTKPREEQYNSTYRVVSVLTVLHQDWLNGKEYKCKVSNKALPAPIEKTISKAKGQPREPQVYTLPPSREEMTKNQVSLTCLVKGFYPSDIAVEWESNGQPENNYKTTPPVLDSDGSFFLYSKLTVDKSRWQQGNVFSCSVMHEALHNHYTQKSLSLSPG

SEQ ID NO: 44 - protein, 226 aa, synthetic construct
DKTHTCPPCPAPELLGGPSVFLFPPKPKDTLMISRTPEVTCVVVDVSHEDPEVKFNWYVDGVEVHNAKTKPREEQYNSTYRVVSVLTVLHQDWLNGKEYKCKVSNKALPAPIEKTISKAKGQPREPQVYTLPPSRXEXTKNQVSLTCLVKGFYPSDIAVEWESNGQPENNYKTTPPVLDSDGSFFLYSKLTVDKSRWQQGNVFSCSVLHEALHSHYTQKSLSLSPG

SEQ ID NO: 45 - protein, 226 aa, synthetic construct
DKTHTCPPCPAPELLGGPSVFLFPPKPKDTLMISRTPEVTCVVVDVSHEDPEVKFNWYVDGVEVHNAKTKPREEQYNSTYRVVSVLTVLHQDWLNGKEYKCKVSNKALPAPIEKTISKAKGQPREPQVYTLPPSRDELTKNQVSLTCLVKGFYPSDIAVEWESNGQPENNYKTTPPVLDSDGSFFLYSKLTVDKSRWQQGNVFSCSVLHEALHSHYTQKSLSLSPG

SEQ ID NO: 46 - protein, 226 aa, synthetic construct
DKTHTCPPCPAPELLGGPSVFLFPPKPKDTLMISRTPEVTCVVVDVSHEDPEVKFNWYVDGVEVHNAKTKPREEQYNSTYRVVSVLTVLHQDWLNGKEYKCKVSNKALPAPIEKTISKAKGQPREPQVYTLPPSREEMTKNQVSLTCLVKGFYPSDIAVEWESNGQPENNYKTTPPVLDSDGSFFLYSKLTVDKSRWQQGNVFSCSVLHEALHSHYTQKSLSLSPG

SEQ ID NO: 47 - protein, 265 aa, synthetic construct
MGWSCIILFLVATATGVHSNVNHKPSNTKVDKKVEPKSSDKTHTCPPCPAPELLGGPSVFLFPPKPKDTLXIXRXPEVTCVVVDVSHEDPEVKFNWYVDGVEVHNAKTKPREEQYNSTYRVVSVLTVLHQDWLNGKEYKCKVSNKALPAPIEKTISKAKGQPREPQVYTLPPSRXEXTKNQVSLTCLVKGFYPSDIAVEWESNGQPENNYKTTPPVLDSDGSFFLYSKLTVDKSRWQQGNVFSCSVXHEALHXHYTQKSLSLSPG

SEQ ID NO: 48 - protein, 266 aa, synthetic construct
MGWSCIILFLVATATGVHSNVNHKPSNTKVDKKVEPKSSDKTHTCPPCPAPELLGGPSVFLFPPKPKDTLMISRTPEVTCVVVDVSHEDPEVKFNWYVDGVEVHNAKTKPREEQYNSTYRVVSVLTVLHQDWLNGKEYKCKVSNKALPAPIEKTISKAKGQPREPQVYTLPPSRDELTKNQVSLTCLVKGFYPSDIAVEWESNGQPENNYKTTPPVLDSDGSFFLYSKLTVDKSRWQQGNVFSCSVMHEALHNHYTQKSLSLSPGK

SEQ ID NO: 49 - protein, 266 aa, synthetic construct
MGWSCIILFLVATATGVHSNVNHKPSNTKVDKKVEPKSSDKTHTCPPCPAPELLGGPSVFLFPPKPKDTLMISRTPEVTCVVVDVSHEDPEVKFNWYVDGVEVHNAKTKPREEQYNSTYRVVSVLTVLHQDWLNGKEYKCKVSNKALPAPIEKTISKAKGQPREPQVYTLPPSREEMTKNQVSLTCLVKGFYPSDIAVEWESNGQPENNYKTTPPVLDSDGSFFLYSKLTVDKSRWQQGNVFSCSVMHEALHNHYTQKSLSLSPGK

SEQ ID NO: 50 - protein, 266 aa, synthetic construct
MGWSCIILFLVATATGVHSNVNHKPSNTKVDKKVEPKSSDKTHTCPPCPAPELLGGPSVFLFPPKPKDTLMISRTPEVTCVVVDVSHEDPEVKFNWYVDGVEVHNAKTKPREEQYNSTYRVVSVLTVLHQDWLNGKEYKCKVSNKALPAPIEKTISKAKGQPREPQVYTLPPSRDELTKNQVSLTCLVKGFYPSDIAVEWESNGQPENNYKTTPPVLDSDGSFFLYSKLTVDKSRWQQGNVFSCSVLHEALHSHYTQKSLSLSPGK

SEQ ID NO: 51 - protein, 266 aa, synthetic construct
MGWSCIILFLVATATGVHSNVNHKPSNTKVDKKVEPKSSDKTHTCPPCPAPELLGGPSVFLFPPKPKDTLMISRTPEVTCVVVDVSHEDPEVKFNWYVDGVEVHNAKTKPREEQYNSTYRVVSVLTVLHQDWLNGKEYKCKVSNKALPAPIEKTISKAKGQPREPQVYTLPPSREEMTKNQVSLTCLVKGFYPSDIAVEWESNGQPENNYKTTPPVLDSDGSFFLYSKLTVDKSRWQQGNVFSCSVLHEALHSHYTQKSLSLSPGK

SEQ ID NO: 52 - protein, 266 aa, synthetic construct
MGWSCIILFLVATATGVHSNVNHKPSNTKVDKKVEPKSSDKTHTCPPCPAPELLGGPSVFLFPPKPKDTLYITREPEVTCVVVDVSHEDPEVKFNWYVDGVEVHNAKTKPREEQYNSTYRVVSVLTVLHQDWLNGKEYKCKVSNKALPAPIEKTISKAKGQPREPQVYTLPPSRDELTKNQVSLTCLVKGFYPSDIAVEWESNGQPENNYKTTPPVLDSDGSFFLYSKLTVDKSRWQQGNVFSCSVMHEALHNHYTQKSLSLSPGK

SEQ ID NO: 53 - protein, 266 aa, synthetic construct
MGWSCIILFLVATATGVHSNVNHKPSNTKVDKKVEPKSSDKTHTCPPCPAPELLGGPSVFLFPPKPKDTLYITREPEVTCVVVDVSHEDPEVKFNWYVDGVEVHNAKTKPREEQYNSTYRVVSVLTVLHQDWLNGKEYKCKVSNKALPAPIEKTISKAKGQPREPQVYTLPPSREEMTKNQVSLTCLVKGFYPSDIAVEWESNGQPENNYKTTPPVLDSDGSFFLYSKLTVDKSRWQQGNVFSCSVMHEALHNHYTQKSLSLSPGK

SEQ ID NO: 54 - protein, 267 aa, synthetic construct
MGWSCIILFLVATATGVHSISAMVRSDKTHTCPPCPAPELLGGPSVFLFPPKPKDTLMISRTPEVTCVVVDVSHEDPEVKFNWYVDGVEVHNAKTKPREEQYNSTYRVVSVLTVLHQDWLNGKEYKCKVSNKALPAPIEKTISKAKGQPREPQVYTLPPSREEMTKNQVSLTCLVKGFYPSDIAVEWESNGQPENNYKTTPPVLDSDGSFFLYSKLTVDKSRWQQGNVFSCSVLHEALHSHYTQKSLSLSPGGGGGSEQKLISEEDL

SEQ ID NO: 55 - protein, 267 aa, synthetic construct
MGWSCIILFLVATATGVHSISAMVRSDKTHTCPPCPAPELLGGPSVFLFPPKPKDTLMISRTPEVTCVVVDVSHEDPEVKFNWYVDGVEVHNAKTKPREEQYNSTYRVVSVLTVLHQDWLNGKEYKCKVSNKALPAPIEKTISKAKGQPREPQVYTLPPSRDELTKNQVSLTCLVKGFYPSDIAVEWESNGQPENNYKTTPPVLDSDGSFFLYSKLTVDKSRWQQGNVFSCSVLHEALHSHYTQKSLSLSPGGGGGSEQKLISEEDL

SEQ ID NO: 56 - protein, 267 aa, synthetic construct
MGWSCIILFLVATATGVHSISAMVRSDKTHTCPPCPAPELLGGPSVFLFPPKPKDTLYITREPEVTCVVVDVSHEDPEVKFNWYVDGVEVHNAKTKPREEQYNSTYRVVSVLTVLHQDWLNGKEYKCKVSNKALPAPIEKTISKAKGQPREPQVYTLPPSREEMTKNQVSLTCLVKGFYPSDIAVEWESNGQPENNYKTTPPVLDSDGSFFLYSKLTVDKSRWQQGNVFSCSVMHEALHNHYTQKSLSLSPGGGGGSEQKLISEEDL

SEQ ID NO: 57 - protein, 267 aa, synthetic construct
MGWSCIILFLVATATGVHSISAMVRSDKTHTCPPCPAPELLGGPSVFLFPPKPKDTLYITREPEVTCVVVDVSHEDPEVKFNWYVDGVEVHNAKTKPREEQYNSTYRVVSVLTVLHQDWLNGKEYKCKVSNKALPAPIEKTISKAKGQPREPQVYTLPPSRDELTKNQVSLTCLVKGFYPSDIAVEWESNGQPENNYKTTPPVLDSDGSFFLYSKLTVDKSRWQQGNVFSCSVMHEALHNHYTQKSLSLSPGGGGGSEQKLISEEDL

SEQ ID NO: 58 - protein, 275 aa, synthetic construct
MGWSCIILFLVATATGVHSEPKSSDKTHTCPPCPAPELLGGPSVFLFPPKPKDTLMISRTPEVTCVVVDVSHEDPEVKFNWYVDGVEVHNAKTKPREEQYNSTYRVVSVLTVLHQDWLNGKEYKCKVSNKALPAPIEKTISKAKGQPREPQVYTLPPSRDELTKNQVSLTCLVKGFYPSDIAVEWESNGQPENNYKTTPPVLDSDGSFFLYSKLTVDKSRWQQGNVFSCSVMHEALHNHYTQKSLSLSPGGGGGSQRNPRLRLIRRHPTLRIPPI

SEQ ID NO: 59 - protein, 275 aa, synthetic construct
MGWSCIILFLVATATGVHSEPKSSDKTHTCPPCPAPELLGGPSVFLFPPKPKDTLMISRTPEVTCVVVDVSHEDPEVKFNWYVDGVEVHNAKTKPREEQYNSTYRVVSVLTVLHQDWLNGKEYKCKVSNKALPAPIEKTISKAKGQPREPQVYTLPPSRDELTKNQVSLTCLVKGFYPSDIAVEWESNGQPENNYKTTPPVLDSDGSFFLYSKLTVDKSRWQQGNVFSCSVLHEALHSHYTQKSLSLSPGGGGGSQRNPRLRLIRRHPTLRIPPI

SEQ ID NO: 60 - protein, 247 aa, synthetic construct
NVNHKPSNTKVDKKVEPKSZDKTHTCPPCPAPELLGGPSVFLFPPKPKDTLXIXRXPEVTCVVVDVSHEDPEVKFNWYVDGVEVHNAKTKPREEQYNSTYRVVSVLTVLHQDWLNGKEYKCKVSNKALPAPIEKTISKAKGQPREPQVYTLPPSRXEXTKNQVSLTCLVKGFYPSDIAVEWESNGQPENNYKTTPPVLDSDGSFFLYSKLTVDKSRWQQGNVFSCSVXHEALHXHYTQKSLSLSPGK

SEQ ID NO: 61 - protein, 247 aa, synthetic construct
NVNHKPSNTKVDKKVEPKSSDKTHTCPPCPAPELLGGPSVFLFPPKPKDTLXIXRXPEVTCVVVDVSHEDPEVKFNWYVDGVEVHNAKTKPREEQYNSTYRVVSVLTVLHQDWLNGKEYKCKVSNKALPAPIEKTISKAKGQPREPQVYTLPPSRXEXTKNQVSLTCLVKGFYPSDIAVEWESNGQPENNYKTTPPVLDSDGSFFLYSKLTVDKSRWQQGNVFSCSVXHEALHXHYTQKSLSLSPGK

SEQ ID NO: 62 - protein, 247 aa, synthetic construct
NVNHKPSNTKVDKKVEPKSSDKTHTCPPCPAPELLGGPSVFLFPPKPKDTLMISRTPEVTCVVVDVSHEDPEVKFNWYVDGVEVHNAKTKPREEQYNSTYRVVSVLTVLHQDWLNGKEYKCKVSNKALPAPIEKTISKAKGQPREPQVYTLPPSRXEXTKNQVSLTCLVKGFYPSDIAVEWESNGQPENNYKTTPPVLDSDGSFFLYSKLTVDKSRWQQGNVFSCSVMHEALHNHYTQKSLSLSPGK

SEQ ID NO: 63 - protein, 247 aa, synthetic construct
NVNHKPSNTKVDKKVEPKSSDKTHTCPPCPAPELLGGPSVFLFPPKPKDTLMISRTPEVTCVVVDVSHEDPEVKFNWYVDGVEVHNAKTKPREEQYNSTYRVVSVLTVLHQDWLNGKEYKCKVSNKALPAPIEKTISKAKGQPREPQVYTLPPSREEMTKNQVSLTCLVKGFYPSDIAVEWESNGQPENNYKTTPPVLDSDGSFFLYSKLTVDKSRWQQGNVFSCSVMHEALHNHYTQKSLSLSPGK

SEQ ID NO: 64 - protein, 247 aa, synthetic construct
NVNHKPSNTKVDKKVEPKSSDKTHTCPPCPAPELLGGPSVFLFPPKPKDTLMISRTPEVTCVVVDVSHEDPEVKFNWYVDGVEVHNAKTKPREEQYNSTYRVVSVLTVLHQDWLNGKEYKCKVSNKALPAPIEKTISKAKGQPREPQVYTLPPSRDELTKNQVSLTCLVKGFYPSDIAVEWESNGQPENNYKTTPPVLDSDGSFFLYSKLTVDKSRWQQGNVFSCSVMHEALHNHYTQKSLSLSPGK

SEQ ID NO: 65 - protein, 247 aa, synthetic construct
NVNHKPSNTKVDKKVEPKSSDKTHTCPPCPAPELLGGPSVFLFPPKPKDTLMISRTPEVTCVVVDVSHEDPEVKFNWYVDGVEVHNAKTKPREEQYNSTYRVVSVLTVLHQDWLNGKEYKCKVSNKALPAPIEKTISKAKGQPREPQVYTLPPSRDELTKNQVSLTCLVKGFYPSDIAVEWESNGQPENNYKTTPPVLDSDGSFFLYSKLTVDKSRWQQGNVFSCSVLHEALHSHYTQKSLSLSPGK

SEQ ID NO: 66 - protein, 247 aa, synthetic construct
NVNHKPSNTKVDKKVEPKSSDKTHTCPPCPAPELLGGPSVFLFPPKPKDTLMISRTPEVTCVVVDVSHEDPEVKFNWYVDGVEVHNAKTKPREEQYNSTYRVVSVLTVLHQDWLNGKEYKCKVSNKALPAPIEKTISKAKGQPREPQVYTLPPSREEMTKNQVSLTCLVKGFYPSDIAVEWESNGQPENNYKTTPPVLDSDGSFFLYSKLTVDKSRWQQGNVFSCSVLHEALHSHYTQKSLSLSPGK

SEQ ID NO: 67 - protein, 247 aa, synthetic construct
NVNHKPSNTKVDKKVEPKSSDKTHTCPPCPAPELLGGPSVFLFPPKPKDTLYITREPEVTCVVVDVSHEDPEVKFNWYVDGVEVHNAKTKPREEQYNSTYRVVSVLTVLHQDWLNGKEYKCKVSNKALPAPIEKTISKAKGQPREPQVYTLPPSRDELTKNQVSLTCLVKGFYPSDIAVEWESNGQPENNYKTTPPVLDSDGSFFLYSKLTVDKSRWQQGNVFSCSVMHEALHNHYTQKSLSLSPGK

SEQ ID NO: 68 - protein, 247 aa, synthetic construct
NVNHKPSNTKVDKKVEPKSSDKTHTCPPCPAPELLGGPSVFLFPPKPKDTLYITREPEVTCVVVDVSHEDPEVKFNWYVDGVEVHNAKTKPREEQYNSTYRVVSVLTVLHQDWLNGKEYKCKVSNKALPAPIEKTISKAKGQPREPQVYTLPPSREEMTKNQVSLTCLVKGFYPSDIAVEWESNGQPENNYKTTPPVLDSDGSFFLYSKLTVDKSRWQQGNVFSCSVMHEALHNHYTQKSLSLSPGK

SEQ ID NO: 69 - protein, 247 aa, synthetic construct
NVNHKPSNTKVDKKVEPKSCDKTHTCPPCPAPELLGGPSVFLFPPKPKDTLYITREPEVTCVVVDVSHEDPEVKFNWYVDGVEVHNAKTKPREEQYNSTYRVVSVLTVLHQDWLNGKEYKCKVSNKALPAPIEKTISKAKGQPREPQVYTLPPSRDELTKNQVSLTCLVKGFYPSDIAVEWESNGQPENNYKTTPPVLDSDGSFFLYSKLTVDKSRWQQGNVFSCSVMHEALHNHYTQKSLSLSPGK

SEQ ID NO: 70 - protein, 247 aa, synthetic construct
NVNHKPSNTKVDKKVEPKSSDKTHTCPPCPAPELLAGPSVFLFPPKPKDTLYITREPEVTCVVVDVSHEDPEVKFNWYVDGVEVHNAKTKPREEQYNSTYRVVSVLTVLHQDWLNGKEYKCKVSNKALPLPEEKTISKAKGQPREPQVYTLPPSRDELTKNQVSLTCLVKGFYPSDIAVEWESNGQPENNYKTTPPVLDSDGSFFLYSKLTVDKSRWQQGNVFSCSVMHEALHNHYTQKSLSLSPGK

SEQ ID NO: 71 - protein, 247 aa, synthetic construct
NVNHKPSNTKVDKKVEPKSCDKTHTCPPCPAPELLGGPSVFLFPPKPKDTLMISRTPEVTCVVVDVSHEDPEVKFNWYVDGVEVHNAKTKPREEQYNSTYRVVSVLTVLHQDWLNGKEYKCKVSNKALPAPIEKTISKAKGQPREPQVYTLPPSRDELTKNQVSLTCLVKGFYPSDIAVEWESNGQPENNYKTTPPVLDSDGSFFLYSKLTVDKSRWQQGNVFSCSVLHEALHSHYTQKSLSLSPGK

SEQ ID NO: 72 - protein, 247 aa, synthetic construct
NVNHKPSNTKVDKKVEPKSCDKTHTCPPCPAPELLGGPSVFLFPPKPKDTLMISRTPEVTCVVVDVSHEDPEVKFNWYVDGVEVHNAKTKPREEQYNSTYRVVSVLTVLHQDWLNGKEYKCKVSNKALPAPIEKTISKAKGQPREPQVYTLPPSRDELTKNQVSLTCLVKGFYPSDIAVEWESNGQPENNYKTTPPVLDSDGSFFLYSKLTVDKSRWQQGNVFSCSVMHEALHNHYTQKSLSLSPGK

SEQ ID NO: 73 - protein, 247 aa, synthetic construct
NVNHKPSNTKVDKKVEPKSCDKTHTCPPCPAPELLGGPSVFLFPPKPKDTLMISRTPEVTCVVVDVSHEDPEVKFNWYVDGVEVHNAKTKPREEQYNSTYRVVSVLTVLHQDWLNGKEYKCKVSNKALPAPIEKTISKAKGQPREPQVYTLPPSREEMTKNQVSLTCLVKGFYPSDIAVEWESNGQPENNYKTTPPVLDSDGSFFLYSKLTVDKSRWQQGNVFSCSVLHEALHSHYTQKSLSLSPGK

SEQ ID NO: 74 - protein, 247 aa, synthetic construct
NVNHKPSNTKVDKKVEPKSCDKTHTCPPCPAPELLAGPSVFLFPPKPKDTLMISRTPEVTCVVVDVSHEDPEVKFNWYVDGVEVHNAKTKPREEQYNSTYRVVSVLTVLHQDWLNGKEYKCKVSNKALPLPEEKTISKAKGQPREPQVYTLPPSRDELTKNQVSLTCLVKGFYPSDIAVEWESNGQPENNYKTTPPVLDSDGSFFLYSKLTVDKSRWQQGNVFSCSVLHEALHSHYTQKSLSLSPGK

SEQ ID NO: 75 - protein, 247 aa, synthetic construct
NVNHKPSNTKVDKKVEPKSCDKTHTCPPCPAPELLAGPSVFLFPPKPKDTLMISRTPEVTCVVVDVSHEDPEVKFNWYVDGVEVHNAKTKPREEQYNSTYRVVSVLTVLHQDWLNGKEYKCKVSNKALPLPEEKTISKAKGQPREPQVYTLPPSREEMTKNQVSLTCLVKGFYPSDIAVEWESNGQPENNYKTTPPVLDSDGSFFLYSKLTVDKSRWQQGNVFSCSVLHEALHSHYTQKSLSLSPGK

SEQ ID NO: 76 - protein, 247 aa, synthetic construct
NVNHKPSNTKVDKKVEPKSSDKTHTCPPCPAPELLAGPSVFLFPPKPKDTLMISRTPEVTCVVVDVSHEDPEVKFNWYVDGVEVHNAKTKPREEQYNSTYRVVSVLTVLHQDWLNGKEYKCKVSNKALPLPEEKTISKAKGQPREPQVYTLPPSRDELTKNQVSLTCLVKGFYPSDIAVEWESNGQPENNYKTTPPVLDSDGSFFLYSKLTVDKSRWQQGNVFSCSVLHEALHSHYTQKSLSLSPGK

SEQ ID NO: 77 - protein, 247 aa, synthetic construct
NVNHKPSNTKVDKKVEPKSSDKTHTCPPCPAPELLAGPSVFLFPPKPKDTLMISRTPEVTCVVVDVSHEDPEVKFNWYVDGVEVHNAKTKPREEQYNSTYRVVSVLTVLHQDWLNGKEYKCKVSNKALPLPEEKTISKAKGQPREPQVYTLPPSREEMTKNQVSLTCLVKGFYPSDIAVEWESNGQPENNYKTTPPVLDSDGSFFLYSKLTVDKSRWQQGNVFSCSVLHEALHSHYTQKSLSLSPGK

SEQ ID NO: 78 - protein, 247 aa, synthetic construct
NVNHKPSNTKVDKKVEPKSSDKTHTCPPCPAPELLGGPSVFLFPPKPKDTLMISRTPEVTCVVVDVSHEDPEVKFNWYVDGVEVHNAKTKPREEQYNSTYRVVSVLTVDHHDWLNGKEYKCKVSNKALPAPIEKTISKAKGQPREPQVYTLPPSRDELTKNQVSLTCLVKGFYPSDIAVEWESNGQPENNYKTTPPVLDSDGSFFLYSKLTVDKSRWQQGNVFSCSVMHEALHSHYTQKSLSLSPGK

SEQ ID NO: 79 - protein, 247 aa, synthetic construct
NVNHKPSNTKVDKKVEPKSSDKTHTCPPCPAPELLGGPSVFLFPPKPKDTLMISRTPEVTCVVVDVSHEDPEVKFNWYVDGVEVHNAKTKPREEQYNSTYRVVSVLTVDHHDWLNGKEYKCKVSNKALPAPIEKTISKAKGQPREPQVYTLPPSREEMTKNQVSLTCLVKGFYPSDIAVEWESNGQPENNYKTTPPVLDSDGSFFLYSKLTVDKSRWQQGNVFSCSVMHEALHSHYTQKSLSLSPGK

SEQ ID NO: 80 - protein, 247 aa, synthetic construct
NVNHKPSNTKVDKKVEPKSCDKTHTCPPCPAPELLGGPSVFLFPPKPKDTLMISRTPEVTCVVVDVSHEDPEVKFNWYVDGVEVHNAKTKPREEQYNSTYRVVSVLTVDHHDWLNGKEYKCKVSNKALPAPIEKTISKAKGQPREPQVYTLPPSRDELTKNQVSLTCLVKGFYPSDIAVEWESNGQPENNYKTTPPVLDSDGSFFLYSKLTVDKSRWQQGNVFSCSVMHEALHSHYTQKSLSLSPGK

SEQ ID NO: 81 - protein, 247 aa, synthetic construct
NVNHKPSNTKVDKKVEPKSCDKTHTCPPCPAPELLGGPSVFLFPPKPKDTLMISRTPEVTCVVVDVSHEDPEVKFNWYVDGVEVHNAKTKPREEQYNSTYRVVSVLTVDHHDWLNGKEYKCKVSNKALPAPIEKTISKAKGQPREPQVYTLPPSREEMTKNQVSLTCLVKGFYPSDIAVEWESNGQPENNYKTTPPVLDSDGSFFLYSKLTVDKSRWQQGNVFSCSVMHEALHSHYTQKSLSLSPGK

SEQ ID NO: 82 - protein, 4 aa, synthetic construct
MVRS

SEQ ID NO: 83 - protein, 7 aa, synthetic construct
ISAMVRS

SEQ ID NO: 84 - protein, 20 aa, synthetic construct
MYRMQLLSCIALSLALVTNS

SEQ ID NO: 85 - protein, 19 aa, synthetic construct
MGWSCIILFLVATATGVHS